European Patent Application EP 4 656 652 A1, published December 3, 2025. Title: NOVEL BRAIN DISEASE THERAPEUTIC AND USE THEREOF. Applicant: Avixgen Inc. Application EP 24747430.7. The sequence listing filed with the application follows.

SEQUENCE LISTING (5 sequences)

SEQ ID NO: 1 - protein, 62 aa, synthetic construct
VKCFNCGKEGHTARNCRAPRKKGHGEGTFTSDLSKQMEEEAVRLFIEWLKNGGPSSGAPPPS

SEQ ID NO: 2 - protein, 55 aa, synthetic construct
ARAPRKKGARAPRKKGHGEGTFTSDLSKQMEEEAVRLFIEWLKNGGPSSGAPPPS

SEQ ID NO: 3 - protein, 39 aa, synthetic construct
HGEGTFTSDLSKQMEEEAVRLFIEWLKNGGPSSGAPPPS

SEQ ID NO: 4 - protein, 23 aa, synthetic construct
VKCFNCGKEGHTARNCRAPRKKG

SEQ ID NO: 5 - protein, 16 aa, synthetic construct
ARAPRKKGARAPRKKG